European Patent Application EP 4 641 196 A1, published October 29, 2025. Title: SYSTEM AND METHOD FOR SCREENING RNA APTAMER. Applicant: CRISMERS BIOTECHNOLOGIES (SHENZHEN) CO., LTD. Application EP 23905840.7, filed December 15, 2023. The sequence listing filed with the application follows.

SEQUENCE LISTING (35 sequences)

SEQ ID NO: 1 - RNA, 20 nt, synthetic construct
  source 1..20: mol_type = other RNA
ctcggtatctagtgcgcact

SEQ ID NO: 2 - RNA, 20 nt, synthetic construct
  source 1..20: mol_type = other RNA
cgtcgactgaaatcctcttc

SEQ ID NO: 3 - RNA, 20 nt, synthetic construct
  source 1..20: mol_type = other RNA
tgttcgttttcgccccgtgg

SEQ ID NO: 4 - RNA, 20 nt, synthetic construct
  source 1..20: mol_type = other RNA
atagtgaatactacagagac

SEQ ID NO: 5 - RNA, 20 nt, synthetic construct
  source 1..20: mol_type = other RNA
tcttacaatgtttagaaggt

SEQ ID NO: 6 - RNA, 20 nt, synthetic construct
  source 1..20: mol_type = other RNA
tgtacagaattctcccgggt

SEQ ID NO: 7 - RNA, 20 nt, synthetic construct
  source 1..20: mol_type = other RNA
attaccgtagtttttgtagt

SEQ ID NO: 8 - skipped

SEQ ID NO: 9 - RNA, 15 nt, synthetic construct
  source 1..15: mol_type = other RNA
ctgcagggccaagtg

SEQ ID NO: 10 - DNA, 100 bp, synthetic construct
  source 1..100: mol_type = other DNA
  misc_feature 41..60: note = n is A, T, C or G.
agcaagttaaaataaggctagtccgttatcaacttggccannnnnnnnnnnnnnnnnnnnctgcagggccaagtggcaccgagtcggtgctttttatcga

SEQ ID NO: 11 - DNA, 40 bp, synthetic construct
  source 1..40: mol_type = other DNA
tatgtttaagagctagaaatagcaagttaaaataaggcta

SEQ ID NO: 12 - DNA, 40 bp, synthetic construct
  source 1..40: mol_type = other DNA
ccatctttgcaaagcttatatcgataaaaagcaccgactc

SEQ ID NO: 13 - RNA, 44 nt, synthetic construct
  source 1..44: mol_type = other RNA
acttggccactcggtatctagtgcgcactctgcagggccaagtg

SEQ ID NO: 14 - RNA, 44 nt, synthetic construct
  source 1..44: mol_type = other RNA
acttggccacgtcgactgaaatcctcttcctgcagggccaagtg

SEQ ID NO: 15 - RNA, 44 nt, synthetic construct
  source 1..44: mol_type = other RNA
acttggccatgttcgttttcgccccgtggctgcagggccaagtg

SEQ ID NO: 16 - RNA, 44 nt, synthetic construct
  source 1..44: mol_type = other RNA
acttggccaatagtgaatactacagagacctgcagggccaagtg

SEQ ID NO: 17 - RNA, 44 nt, synthetic construct
  source 1..44: mol_type = other RNA
acttggccatcttacaatgtttagaaggtctgcagggccaagtg

SEQ ID NO: 18 - RNA, 44 nt, synthetic construct
  source 1..44: mol_type = other RNA
acttggccatgtacagaattctcccgggtctgcagggccaagtg

SEQ ID NO: 19 - RNA, 44 nt, synthetic construct
  source 1..44: mol_type = other RNA
acttggccaattaccgtagtttttgtagtctgcagggccaagtg

SEQ ID NO: 20 - RNA, 82 nt, synthetic construct
  source 1..82: mol_type = other RNA
gcttctggactgcgatgggagcacgaaacgtcgtggcgcaattgggtggggaaagtccttaaaagagggccaccacagaagc

SEQ ID NO: 21 - DNA, 369 bp, synthetic construct
  source 1..369: mol_type = other DNA
tttcccatgattccttcatatttgcatatacgatacaaggctgttagagagataattagaattaatttgactgtaaacacaaagatattagtacaaaatacgtgacgtagaaagtaataatttcttgggtagtttgcagttttaaaattatgttttaaaatggactatcatatgcttaccgtaacttgaaagtatttcgatttcttggctttatatatcttgtggaaaggacgaaacaccgatctagatacgactcactatgtttaagagctagaaatagcaagttaaaataaggctagtccgttatcaacttggccaggagacggacgtctcactgcagggccaagtggcaccgagtcggtgcttttt

SEQ ID NO: 22 - protein, 692 aa, synthetic construct
  REGION 223..236: note = linker
RVQPTESIVRFPNITNLCPFGEVFNATRFASVYAWNRKRISNCVADYSVLYNSASFSTFKCYGVSPTKLNDLCFTNVYADSFVIRGDEVRQIAPGQTGKIADYNYKLPDDFTGCVIAWNSNNLDSKVGGNYNYLYRLFRKSNLKPFERDISTEIYQAGSTPCNGVEGFNCYFPLQSYGFQPTNGVGYQPYRVVVLSFELLHAPATVCGPKKSTNLVKNKCVNFEFGGSGGSGGSDRGSDALDDFDLDMLGSDALDDFDLDMLGSDALDDFDLDMLGSDALDDFDLDMLGSSGGGGGSAINSQYLPDTDDRHRIEEKRKRTYETFKSIMKKSPFSGPTDPRPPPRRIAVPSRSSASVPKPAPQPYPFTSSLSTINYDEFPTMVFPSGQISQASALAPAPPQVLPQAPAPAPAPAMVSALAQAPAPVPVLAPGPPQAVAPPAPKPTQAGEGTLSEALLQLQFDDEDLGALLGNSTDPAVFTDLASVDNSEFQQLLNQGIPVAPHTTEPMLMEYPEAITRLVTGAQRPPDPAPAPLGAPGLPNGLLSGDEDFSSIADMDFSALLSGGGGGSGFSVDTSALLDLFSPSVTVPDMSLPDLDSSLASIQELLSPQEPPRPPEAENSSPDSGKQLVHYTAQPLFLLDPGSVDTGSNDLPVLFELGEGSYFSEGDGFAEDPTISLLTGSEPPKAKDPTVS

SEQ ID NO: 23 - protein, 1371 aa, synthetic construct
MDKKYSIGLAIGTNSVGWAVITDEYKVPSKKFKVLGNTDRHSIKKNLIGALLFDSGETAEATRLKRTARRRYTRRKNRICYLQEIFSNEMAKVDDSFFHRLEESFLVEEDKKHERHPIFGNIVDEVAYHEKYPTIYHLRKKLVDSTDKADLRLIYLALAHMIKFRGHFLIEGDLNPDNSDVDKLFIQLVQTYNQLFEENPINASGVDAKAILSARLSKSRRLENLIAQLPGEKKNGLFGNLIALSLGLTPNFKSNFDLAEDAKLQLSKDTYDDDLDNLLAQIGDQYADLFLAAKNLSDAILLSDILRVNTEITKAPLSASMIKRYDEHHQDLTLLKALVRQQLPEKYKEIFFDQSKNGYAGYIDGGASQEEFYKFIKPILEKMDGTEELLVKLNREDLLRKQRTFDNGSIPHQIHLGELHAILRRQEDFYPFLKDNREKIEKILTFRIPYYVGPLARGNSRFAWMTRKSEETITPWNFEEVVDKGASAQSFIERMTNFDKNLPNEKVLPKHSLLYEYFTVYNELTKVKYVTEGMRKPAFLSGEQKKAIVDLLFKTNRKVTVKQLKEDYFKKIECFDSVEISGVEDRFNASLGTYHDLLKIIKDKDFLDNEENEDILEDIVLTLTLFEDREMIEERLKTYAHLFDDKVMKQLKRRRYTGWGRLSRKLINGIRDKQSGKTILDFLKSDGFANRNFMQLIHDDSLTFKEDIQKAQVSGQGDSLHEHIANLAGSPAIKKGILQTVKVVDELVKVMGRHKPENIVIEMARENQTTQKGQKNSRERMKRIEEGIKELGSQILKEHPVENTQLQNEKLYLYYLQNGRDMYVDQELDINRLSDYDVDAIVPQSFLKDDSIDNKVLTRSDKNRGKSDNVPSEEVVKKMKNYWRQLLNAKLITQRKFDNLTKAERGGLSELDKAGFIKRQLVETRQITKHVAQILDSRMNTKYDENDKLIREVKVITLKSKLVSDFRKDFQFYKVREINNYHHAHDAYLNAVVGTALIKKYPKLESEFVYGDYKVYDVRKMIAKSEQEIGKATAKYFFYSNIMNFFKTEITLANGEIRKRPLIETNGETGEIVWDKGRDFATVRKVLSMPQVNIVKKTEVQTGGFSKESILPKRNSDKLIARKKDWDPKKYGGFDSPTVAYSVLVVAKVEKGKSKKLKSVKELLGITIMERSSFEKNPIDFLEAKGYKEVKKDLIIKLPKYSLFELENGRKRMLASAGELQKGNELALPSKYVNFLYLASHYEKLKGSPEDNEQKQLFVEQHKHYLDEIIEQISEFSKRVILADANLDKVLSAYNKHRDKPIREQAENIIHLFTLTNLGAPAAFKYFDTTIDRKRYTSTKEVLDATLIHQSITGLYETRIDLSQLGGDEGA

SEQ ID NO: 24 - protein, 530 aa, synthetic construct
MAKNTITKTLKLRIVRPYNSAEVEKIVADEKNNREKIALEKNKDKVKEACSKHLKVAAYCTTQVERNACLFCKARKLDDKFYQKLRGQFPDAVFWQEISEIFRQLQKQAAEIYNQSLIELYYEIFIKGKGIANASSVEHYLSRVCYRRAAELFKNAAIASGLRSKIKSNFRLKELKNMKSGLPTTKSDNFPIPLVKQKGGQYTGFEISNHNSDFIIKIPFGRWQVKKEIDKYRPWEKFDFEQVQKSPKPISLLLSTQRRKRNKGWSKDEGTEAEIKKVMNGDYQTSYIEVKRGSKICEKSAWMLNLSIDVPKIDKGVDPSIIGGIAVGVRSPLVCAINNAFSRYSISDNDLFHFNKKMFARRRILLKKNRHKRAGHGAKNKLKPITILTEKSERFRKKLIERWACEIADFFIKNKVGTVQMENLESMKRKEDSYFNIRLRGFWPYAEMQNKIEFKLKQYGIEIRKVAPNNTSKTCSKCGHLNNYFNFEYRKKNKFPHFKCEKCNFKENAAYNAALNISNPKLKSTKERPA

SEQ ID NO: 25 - DNA, 42 bp, synthetic construct
  source 1..42: mol_type = other DNA
ggcggtagtggtggtgaattcagagtccaaccaacagaatct

SEQ ID NO: 26 - DNA, 46 bp, synthetic construct
  source 1..46: mol_type = other DNA
accgccagagccaccgaattcgaaattgacacatttgtttttaacc

SEQ ID NO: 27 - DNA, 32 bp, synthetic construct
  source 1..32: mol_type = other DNA
tagagggtatataatggaagctcgacttccag

SEQ ID NO: 28 - DNA, 32 bp, synthetic construct
  source 1..32: mol_type = other DNA
tagagggtatataatggaagctcgaattccag

SEQ ID NO: 29 - DNA, 63 bp, synthetic construct
  source 1..63: mol_type = other DNA
ttcgcatattaaggtgacgcgtgtggcctcgaacaccgagcgaccctgcagcgacccgcttaa

SEQ ID NO: 30 - DNA, 39 bp, synthetic construct
  source 1..39: mol_type = other DNA
ggtaggcgtgtacggtgggaggtctatataagcagagct

SEQ ID NO: 31 - DNA, 197 bp, synthetic construct
  source 1..197: mol_type = other DNA
agtagaagctctcgatcgcgaatctgttcccggggatcctctagagtcgacctgcagggccagcccaggctccggggcacgtaaaagcggggctgtgagaccggagagcacggagcgaccagccagggctgagctgcggagacggtgagcagggctgtgcgggcagccaagcttggcattccggtactgttggtaaa

SEQ ID NO: 32 - DNA, 23 bp, synthetic construct
  source 1..23: mol_type = other DNA
atctagatacgactcactatagg

SEQ ID NO: 33 - DNA, 351 bp, synthetic construct
  source 1..351: mol_type = other DNA
atctagatacgactcactataggcaaagctctaatctagatacgactcactataggaaaggaagcagccacatctagatacgactcactataggataacgttagatctagatacgactcactatagggtgaagtagtctttgcggtaggagacctattcgagatctagatacgactcactataggcaaagctctaatctagatacgactcactataggaaaggaagcagccacatctagatacgactcactataggataacgttagatctagatacgactcactatagggtgaagtagtctttgcggtaatctagatacgactcactataggatccacgtatgtcgagggt

SEQ ID NO: 34 - DNA, 27 bp, synthetic construct
  source 1..27: mol_type = other DNA
tttgctccctatcagtgatagagaacg

SEQ ID NO: 35 - DNA, 353 bp, synthetic construct
  source 1..353: mol_type = other DNA
tttgctccctatcagtgatagagaacgcaaagctctatttgctccctatcagtgatagagaacgaaaggaagcagccactttgctccctatcagtgatagagaacgataacgttagtttgctccctatcagtgatagagaacggtgaagtagtctttgcggtatttgctccctatcagtgatagagaacgcaaagctctatttgctccctatcagtgatagagaacgaaaggaagcagccactttgctccctatcagtgatagagaacgataacgttagtttgctccctatcagtgatagagaacggtgaagtagtctttgcggtatttgctccctatcagtgatagagaacg